European Patent Specification EP 3 624 837 B1, published July 30, 2025. Title: ANTI-FGFR2 ANTIBODIES IN COMBINATION WITH CHEMOTHERAPY AGENTS IN CANCER TREATMENT. Applicant: Five Prime Therapeutics, Inc. The sequence listing filed with the application follows.

SEQUENCE LISTING (22 sequences)

SEQ ID NO: 1 - protein, 801 aa, Homo sapiens
RPSFSLVEDTTLEPEEPPTKYQISQPEVYVAAPGESLEVRCLLKDAAVISWTKDGVHLGPNNRTVLIGEYLQIKGATPRDSGLYACTASRTVDSETWYFMVNVTDAISSGDDEDDTDGAEDFVSENSNNKRAPYWTNTEKMEKRLHAVPAANTVKFRCPAGGNPMPTMRWLKNGKEFKQEHRIGGYKVRNQHWSLIMESVVPSDKGNYTCVVENEYGSINHTYHLDVVERSPHRPILQAGLPANASTVVGGDVEFVCKVYSDAQPHIQWIKHVEKNGSKYGPDGLPYLKVLKHSGINSSNAEVLALFNVTEADAGEYICKVSNYIGQANQSAWLTVLPKQQAPGREKEITASPDYLEIAIYCIGVFLIACMVVTVILCRMKNTTKKPDFSSQPAVHKLTKRIPLRRQVTVSAESSSSMNSNTPLVRITTRLSSTADTPMLAGVSEYELPEDPKWEFPRDKLTLGKPLGEGCFGQVVMAEAVGIDKDKPKEAVTVAVKMLKDDATEKDLSDLVSEMEMMKMIGKHKNIINLLGACTQDGPLYVIVEYASKGNLREYLRARRPPGMEYSYDINRVPEEQMTFKDLVSCTYQLARGMEYLASQKCIHRDLAARNVLVTENNVMKIADFGLARDINNIDYYKKTTNGRLPVKWMAPEALFDRVYTHQSDVWSFGVLMWEIFTLGGSPYPGIPVEELFKLLKEGHRMDKPANCTNELYMMMRDCWHAVPSQRPTFKQLVEDLDRILTLTTNEEYLDLSQPLEQYSPSYPDTRSSCSSGDDSVFSPDPMPYEPCLPQYPHINGSVKT

SEQ ID NO: 2 - protein, 444 aa, Artificial Sequence
  alpha-FGFR2b heavy chain
  MISC_FEATURE (294)..(294): Asn297
QVQLVQSGAEVKKPGSSVKVSCKASGYIFTTYNVHWVRQAPGQGLEWIGSIYPDNGDTSYNQNFKGRATITADKSTSTAYMELSSLRSEDTAVYYCARGDFAYWGQGTLVTVSSASTKGPSVFPLAPSSKSTSGGTAALGCLVKDYFPEPVTVSWNSGALTSGVHTFPAVLQSSGLYSLSSVVTVPSSSLGTQTYICNVNHKPSNTKVDKRVEPKSCDKTHTCPPCPAPELLGGPSVFLFPPKPKDTLMISRTPEVTCVVVDVSHEDPEVKFNWYVDGVEVHNAKTKPREEQYNSTYRVVSVLTVLHQDWLNGKEYKCKVSNKALPAPIEKTISKAKGQPREPQVYTLPPSREEMTKNQVSLTCLVKGFYPSDIAVEWESNGQPENNYKTTPPVLDSDGSFFLYSKLTVDKSRWQQGNVFSCSVMHEALHNHYTQKSLSLSPGK

SEQ ID NO: 3 - protein, 214 aa, Artificial Sequence
  Anti-FGFR2b light chain
DIQMTQSPSSLSASVGDRVTITCKASQGVSNDVAWYQQKPGKAPKLLIYSASYRYTGVPSRFSGSGSGTDFTFTISSLQPEDIATYYCQQHSTTPYTFGQGTKLEIKRTVAAPSVFIFPPSDEQLKSGTASVVCLLNNFYPREAKVQWKVDNALQSGNSQESVTEQDSKDSTYSLSSTLTLSKADYEKHKVYACEVTHQGLSSPVTKSFNRGEC

SEQ ID NO: 4 - protein, 114 aa, Artificial Sequence [sequence omitted]

SEQ ID NO: 5 - protein, 107 aa, Artificial Sequence [sequence omitted]

SEQ ID NO: 6 - protein, 5 aa, Artificial Sequence
  Anti-FGFR2b heavy chain (HC) HVR1
TYNVH

SEQ ID NO: 7 - protein, 17 aa, Artificial Sequence
  Anti-FGFR2b HC HVR2
SIYPDNGDTSYNQNFKG

SEQ ID NO: 8 - protein, 5 aa, Artificial Sequence
  Anti-FGFR2b HC HVR3
GDFAY

SEQ ID NO: 9 - protein, 11 aa, Artificial Sequence
  Anti-FGFR2b light chain (LC) HVR1
KASQGVSNDVA

SEQ ID NO: 10 - protein, 7 aa, Artificial Sequence
  Anti-FGFR2b LC HVR2
SASYRYT

SEQ ID NO: 11 - protein, 9 aa, Artificial Sequence
  Anti-FGFR2b LC HVR3
QQHSTTPYT

SEQ ID NO: 12 - protein, 444 aa, Artificial Sequence
  Anti-FGFR2b N297Q heavy chain
  MISC_FEATURE (294)..(294): N297Q
QVQLVQSGAEVKKPGSSVKVSCKASGYIFTTYNVHWVRQAPGQGLEWIGSIYPDNGDTSYNQNFKGRATITADKSTSTAYMELSSLRSEDTAVYYCARGDFAYWGQGTLVTVSSASTKGPSVFPLAPSSKSTSGGTAALGCLVKDYFPEPVTVSWNSGALTSGVHTFPAVLQSSGLYSLSSVVTVPSSSLGTQTYICNVNHKPSNTKVDKRVEPKSCDKTHTCPPCPAPELLGGPSVFLFPPKPKDTLMISRTPEVTCVVVDVSHEDPEVKFNWYVDGVEVHNAKTKPREEQYQSTYRVVSVLTVLHQDWLNGKEYKCKVSNKALPAPIEKTISKAKGQPREPQVYTLPPSREEMTKNQVSLTCLVKGFYPSDIAVEWESNGQPENNYKTTPPVLDSDGSFFLYSKLTVDKSRWQQGNVFSCSVMHEALHNHYTQKSLSLSPGK

SEQ ID NO: 13 - protein, 800 aa, Homo sapiens
RPSFSLVEDTTLEPEEPPTKYQISQPEVYVAAPGESLEVRCLLKDAAVISWTKDGVHLGPNNRTVLIGEYLQIKGATPRDSGLYACTASRTVDSETWYFMVNVTDAISSGDDEDDTDGAEDFVSENSNNKRAPYWTNTEKMEKRLHAVPAANTVKFRCPAGGNPMPTMRWLKNGKEFKQEHRIGGYKVRNQHWSLIMESVVPSDKGNYTCVVENEYGSINHTYHLDVVERSPHRPILQAGLPANASTVVGGDVEFVCKVYSDAQPHIQWIKHVEKNGSKYGPDGLPYLKVLKAAGVNTTDKEIEVLYIRNVTFEDAGEYTCLAGNSIGISFHSAWLTVLPAPGREKEITASPDYLEIAIYCIGVFLIACMVVTVILCRMKNTTKKPDFSSQPAVHKLTKRIPLRRQVTVSAESSSSMNSNTPLVRITTRLSSTADTPMLAGVSEYELPEDPKWEFPRDKLTLGKPLGEGCFGQVVMAEAVGIDKDKPKEAVTVAVKMLKDDATEKDLSDLVSEMEMMKMIGKHKNIINLLGACTQDGPLYVIVEYASKGNLREYLRARRPPGMEYSYDINRVPEEQMTFKDLVSCTYQLARGMEYLASQKCIHRDLAARNVLVTENNVMKIADFGLARDINNIDYYKKTTNGRLPVKWMAPEALFDRVYTHQSDVWSFGVLMWEIFTLGGSPYPGIPVEELFKLLKEGHRMDKPANCTNELYMMMRDCWHAVPSQRPTFKQLVEDLDRILTLTTNEEYLDLSQPLEQYSPSYPDTRSSCSSGDDSVFSPDPMPYEPCLPQYPHINGSVKT

SEQ ID NO: 14 - protein, 356 aa, Homo sapiens
RPSFSLVEDTTLEPEEPPTKYQISQPEVYVAAPGESLEVRCLLKDAAVISWTKDGVHLGPNNRTVLIGEYLQIKGATPRDSGLYACTASRTVDSETWYFMVNVTDAISSGDDEDDTDGAEDFVSENSNNKRAPYWTNTEKMEKRLHAVPAANTVKFRCPAGGNPMPTMRWLKNGKEFKQEHRIGGYKVRNQHWSLIMESVVPSDKGNYTCVVENEYGSINHTYHLDVVERSPHRPILQAGLPANASTVVGGDVEFVCKVYSDAQPHIQWIKHVEKNGSKYGPDGLPYLKVLKAAGVNTTDKEIEVLYIRNVTFEDAGEYTCLAGNSIGISFHSAWLTVLPAPGREKEITASPDYLE

SEQ ID NO: 15 - protein, 119 aa, Artificial Sequence
  Anti-FGFR2 Gal-FR22 heavy chain variable region
QVQLKQSGPGLVQPSQSLSITCTVSGFSLTSFGVHWVRQSPGKGLEWLGVIWSGGSTDYNADFRSRLSISKDNSKSQIFFKMNSLQPDDTIAYCANFYYGYDDYVMDYWGQGTSVTVSS

SEQ ID NO: 16 - protein, 5 aa, Artificial Sequence
  Anti-FGFR2 Gal-FR22 heavy chain CDR1
SFGVH

SEQ ID NO: 17 - protein, 16 aa, Artificial Sequence
  Anti-FGFR2 Gal-FR22 heavy chain CDR2
VIWSGGSTDYNADFRS

SEQ ID NO: 18 - protein, 12 aa, Artificial Sequence
  Anti-FGFR2 Gal-FR22 heavy chain CDR3
FYYGYDDYVMDY

SEQ ID NO: 19 - protein, 107 aa, Artificial Sequence
  Anti-FGFR2 Gal-FR22 light chain variable region
DIQMTQSPSSLSASLGGRVTITCKASQDIKNYIAWYQHKPGKSPRLLIHYTSTLQPGVPSRFSGSGSGRDYSFSISNLEPEDIATYYCLQYDDDLYMFGGGTKLDIK

SEQ ID NO: 20 - protein, 11 aa, Artificial Sequence
  Anti-FGFR2 Gal-FR22 light chain CDR1
KASQDIKNYIA

SEQ ID NO: 21 - protein, 7 aa, Artificial Sequence
  Anti-FGFR2 Gal-FR22 light chain CDR2
YTSTLQP

SEQ ID NO: 22 - protein, 8 aa, Artificial Sequence
  Anti-FGFR2 Gal-FR22 light chain CDR3
LQYDDLYM